European Patent Specification EP 4 240 351 B1, published August 27, 2025. Title: COMPOSITION FOR ENHANCING INTRA-CELLULAR NITRIC OXIDE GENERATION. Applicant: INSTITUTE OF LIFE SCIENCES TRANSLATIONAL HEALTH SCIENCES AND TECHNOLOGY INSTITUTE. Application 202031050500. The sequence listing filed with the application follows.

SEQUENCE LISTING (28 sequences)

SEQ ID NO: 1 - DNA, 21 bp, Human
tgccaccttttgacagtgatg

SEQ ID NO: 2 - DNA, 20 bp, Human
aaggtccacgggaaagacac

SEQ ID NO: 3 - DNA, 20 bp, Human
tccagttgccttcttgggac

SEQ ID NO: 4 - DNA, 23 bp, Human
gccattgcacaactcttttctca

SEQ ID NO: 5 - DNA, 20 bp, Human
ggttgccaagccttatcgga

SEQ ID NO: 6 - DNA, 20 bp, Human
aatcgatgacagcgcctcag

SEQ ID NO: 7 - DNA, 18 bp, Human
cagagggaagagttccca

SEQ ID NO: 8 - DNA, 20 bp, Human
ccttggtctggtaggagacg

SEQ ID NO: 9 - DNA, 20 bp, Human
gagaagaaacacagcccctg

SEQ ID NO: 10 - DNA, 20 bp, Human
tcagtcttcccagcacattg

SEQ ID NO: 11 - DNA, 17 bp, Human
gtgcaggaacctctgac

SEQ ID NO: 12 - DNA, 20 bp, Human
cttctgctctgaccacctcc

SEQ ID NO: 13 - DNA, 20 bp, Human
gactcatctgctgcatggaa

SEQ ID NO: 14 - DNA, 20 bp, Human
tgttgcatcacacaggcttt

SEQ ID NO: 15 - DNA, 20 bp, Human
tccatcagcagctcaatgac

SEQ ID NO: 16 - DNA, 20 bp, Human
tatgtcctcacagccagcag

SEQ ID NO: 17 - DNA, 20 bp, Human
ctgcctgaaggacagaaagg

SEQ ID NO: 18 - DNA, 20 bp, Human
atgcagaacacagagggctt

SEQ ID NO: 19 - DNA, 24 bp, Human
tctggagcatctcttggatggcaa

SEQ ID NO: 20 - DNA, 24 bp, Human
tccagctccaagaaaggacgaaca

SEQ ID NO: 21 - DNA, 22 bp, Human
gattactgctctggctcctagc

SEQ ID NO: 22 - DNA, 22 bp, Human
gactcatcgtactcctgcttgc

SEQ ID NO: 23 - DNA, 912 bp, Human
catatgacgcgccacggcaaaaattgcacggcgggtgcggtttatacctaccacgaaaaaaaaaaagacacggcagcaagcggctacggcacccaaaacattcgtctgagccgcgatgcagtgaaagattttgactgctgttgcctgagcctgcaaccgtgccatgatccggtggttacgccggacggctatctgtacgaacgtgaagctattctggaatatatcctgcatcagaaaaaagaaattgcgcgtcaaatgaaagcctacgaaaaacagcgcggcacccgtcgcgaagaacagaaagaactgcaacgtgcggccagccaagatcatgtccgcggttttctggaaaaagaaagcgccatcgtgtctcgcccgctgaatccgttcaccgcaaaagctctgagcggtacgagcccggatgatgttcagccgggtccgagcgtcggtccgccgagcaaagataaagacaaagtgctgccgagcttttggattccgagcctgaccccggaagcgaaagccacgaaactggaaaaaccgagccgtaccgtgacgtgcccgatgagcggcaaaccgctgcgcatgtctgatctgaccccggttcacttcacgccgctggatagctctgttgaccgtgtcggtctgattacccgtagcgaacgctatgtgtgcgcggttacccgtgacagcctgagcaatgcaacgccgtgcgctgttctgcgcccgtctggtgcggttgtgaccctggaatgcgtcgaaaaactgatccgtaaagatatggttgatccggtgaccggcgataaactgacggatcgtgacattatcgttctgcaacgtggcggcaccggtttcgcaggcagcggtgtgaaactgcaagctgaaaaaagccgcccggttatgcaggcgctcgag

SEQ ID NO: 24 - DNA, 1284 bp, Human
catatgccgcgccatgttcgtatcaaaaattggggtagcggtatgacgtttcaggatacgctgcatcataaagcaaaaggcatcctgacctgccgtagcaaatcttgcctgggtagcatcatgaccccgaaaagcctgacgcgtggcccgcgcgataaaccgaccccgccggatgaactgctgccgcaggcgatcgaatttgtgaaccagtactacggtagcttcaaagaagccaaaattgaagaacatctggcgcgcgttgaagccgtcaccaaagaaatcgaaaccacgggcacctaccagctgacgggcgatgaactgatttttgcaacgaaacaggcgtggcgtaacgcgccgcgttgcattggccgtatccagtggagcaatctgcaggtctttgatgcccgcagctgcagcaccgcacgtgaaatgttcgaacatatctgccgtcatgttcgctatagcaccaacaatggtaacattcgtagcgcgatcacggtgtttccgcagcgcagcgatggcaaacatgatttccgtgtttggaatgcacagctgattcgctacgcgggttatcagatgccggatggcagcatccgcggtgatccggcaaacgtggaatttacccagctgtgcatcgatctgggttggaaaccgaaatatggccgtttcgatgtggttccgctggttctgcaggccaatggccgcgatccggaactgtttgaaattccgccggatctggtgctggaagttgcaatggaacatccgaaatacgaatggttccgtgaactggaactgaaatggtatgcactgccggcagttgcaaacatgctgctggaagtcggcggtctggaatttccgggttgcccgttcaatggctggtacatgggcaccgaaattggcgtccgcgatttttgcgatgtgcagcgttataacatcctggaagaagtgggtcgtcgcatgggcctggaaacgcataaactggccagcctgtggaaagatcaggcagtcgtggaaattaacatcgcagtcctgcattcttttcagaaacagaatgtgaccattatggatcatcatagcgcggccgaatctttcatgaaatacatgcagaacgaatatcgttctcgcggcggttgcccggcggattggatttggctggttccgccgatgagcggcagcatcaccccggtttttcatcaggaaatgctgaactatgtcctgagcccgttctattactatcaggtggaagcctggaaaacgcatgtttggcaggatgaaaaactcgag

SEQ ID NO: 25 - protein, 14 aa, Human
TGDELIFATKQAWR

SEQ ID NO: 26 - protein, 18 aa, Human
NQYYGSFKEAKIEEHLAR

SEQ ID NO: 27 - protein, 34 aa, Human
GWKPKYGRFDVVPLVLQANGRDPELFEIPPDLVL

SEQ ID NO: 28 - protein, 33 aa, Human
NLQVFDARSCSTAREMFEHICRHVRYSTNNGNI